European Patent Application EP 4 400 579 A1, published July 17, 2024. Title: 乳酸菌、乳酸菌スターター、発酵乳、発酵乳の製造方法、及び乳酸菌のスクリーニング方法. Applicant: Meiji Co., Ltd. Application JP. The sequence listing filed with the application follows.

SEQUENCE LISTING (26 sequences)

SEQ ID NO: 1 - DNA, 708 bp, Streptococcus thermophilus
  source 1..708: mol_type = genomic DNA
gtggaaactacaagtaatccaaccgtctcattatttgggattgattttgacttgacgatccttgccatgtctctcttgacagtaattatcgtttttggagtggttttttggtcaagtcgtgatatgaccattaaaccaaagggaaaacaaaatgtactcgagttcatctatgaatttgtgaacaacaccatttctcaaagtcttggaaaattcacaaaaaattatagtttgctcttgtttgtaattttcacctttgtgtttacagcaaacaacttaggtttgcttgtatctgttaaaagtgagcattacaatttttggtcttctccaacatcgaatttcggtgttactatcactctttctttgattattaccctcgttagtcatattgaggggattcgtaaaaaagggtttaaaggctatctcaaaggttacctttcaccatacccagctatgctcccaatgaacattttggaagaatttaccaaccttgcatcattggccttgcgtttgtttggtaacatttattctggtgaggtactaattgacttgattcttcaattagtgaaatggtctgtttttgcagcacctatgtcctttgctttgaaccttgtctgggttgccttttcagcttttattgggttcattcaagcctatgtctttattatcctaagttctaactacattggtgataaagtcaacgaagaataa

SEQ ID NO: 2 - protein, 235 aa, Streptococcus thermophilus
VETTSNPTVSLFGIDFDLTILAMSLLTVIIVFGVVFWSSRDMTIKPKGKQNVLEFIYEFVNNTISQSLGKFTKNYSLLLFVIFTFVFTANNLGLLVSVKSEHYNFWSSPTSNFGVTITLSLIITLVSHIEGIRKKGFKGYLKGYLSPYPAMLPMNILEEFTNLASLALRLFGNIYSGEVLIDLILQLVKWSVFAAPMSFALNLVWVAFSAFIGFIQAYVFIILSSNYIGDKVNEE

SEQ ID NO: 3 - DNA, 498 bp, Streptococcus thermophilus
  source 1..498: mol_type = genomic DNA
atgtcattactgattaatagtacgacacttggtaatatcattattacgctcggctcagtttttctcttgtattacctcattcgtaaattcgcatgggatcaaattacaggaatctttgtcgctcgtgaaaagaaaattgccacagatattgatagtgctgaaaatgctcgtcaagaagcagaaatcttggtacaaaaacgtcaagaggagttagctgccgctcgcacagaagcaactcagattattgatgaggccaagaaaactggtaaaactaaagagtcaaaaatcattgcagaagcatatgatgaagctaaacgcttgaaagagaaagcaaatcaagatatcgcccaaagctgggtggaagcacttgctggcgttaaaggtgaggttgctgacttgactgtccttttggcagaaaaagtcatgaaacaaaaccttgatgcaaaagcgcaatctgacttgattgatagctatcttgatcaattaggagatgcttaa

SEQ ID NO: 4 - protein, 165 aa, Streptococcus thermophilus
MSLLINSTTLGNIIITLGSVFLLYYLIRKFAWDQITGIFVAREKKIATDIDSAENARQEAEILVQKRQEELAAARTEATQIIDEAKKTGKTKESKIIAEAYDEAKRLKEKANQDIAQSWVEALAGVKGEVADLTVLLAEKVMKQNLDAKAQSDLIDSYLDQLGDA

SEQ ID NO: 5 - DNA, 198 bp, Streptococcus thermophilus
  source 1..198: mol_type = genomic DNA
atgaatttaactatcttaggcctcggtttggccgttatgggtgtatctattggtgagggtatcctcgttgccaatatcgctaaggctgcagctcgccaacctgagatgtttagtaaacttcaaacattgatgtttactggtgttgccttcatcgaaggtactttcttcgtattgtttgcccttagctacattgtctaa

SEQ ID NO: 6 - protein, 65 aa, Streptococcus thermophilus
MNLTILGLGLAVMGVSIGEGILVANIAKAAARQPEMFSKLQTLMFTGVAFIEGTFFVLFALSYIV

SEQ ID NO: 7 - DNA, 1506 bp, Streptococcus thermophilus
  source 1..1506: mol_type = genomic DNA
ttggcaattaatgcacaagaaattagcgctttaattaaaaagcaaattgaaaacttccagccaaattttgacgtcacagaaactggtgtagtcacttatatcggtgatggtattgcccgtgctcgtggacttgataatgccatgagtggagaacttctcgaattttcaaatggtgtcttcggtatggctcaaaaccttgagtctaatgacgttggtatcattattcttggagatttttatacaattcgtgaaggtgatgaggttaaacgtactggtaaaatcatggaagtgccagtaggtgaagctcttattggtcgtgtcgtaaacccacttggtcaaccaattgatggtcttggagatatcaagacaactgcaactcgtccagttgaagcacctgcaccaggcgttatgcaacgtaaatcagtttctgaaccactccaaactggtcttaaagcggttgatgctttggttccaattggacgtggtcaacgtgagttaatcatcggtgaccgtcaaacaggtaaaacatctgttgcgattgatgcaattttgaaccaaaaaggacaagatgtgatttgtatctatgttgctattggtcaaaaagaatcaactgtccgtacacaagttgaatcacttcgtaaacatggtgctcttgattacacaatcgttgtgactgcctcagcatcacaaccatcaccattgctttacatcgcgccttacgctggtgttgcaatggctgaagagttcatgtataacggaaaacatgtcttgattgtttatgatgatttgtctaagcaagccgtggcttaccgtgaactttcattgcttctccgtcgtccaccaggtcgtgaagcctacccaggggatgtattctatctccactcacgtcttttggaacgttcagctaagctttcagatgatcttggtggcggttcaattactgccttgccaatcatccaaacacaagcaggagatatctcagcttatattgcgacaaacgttatttctatcacagatggacaaatcttcttgcaagaaaatcttttcaactcaggtattcgtcctgcgattgatgctggttcttcagtatcacgtgttggtggttcagcacaaatcaaagcaatgaagaaagttgctggtacccttcgtcttgacttggcttcttaccgtgaacttgaagcctttacacaattcggttctgatttggatgccgcaacacaagctaaacttaatcgtggacgtcgtacagttgaagtgcttaaacaaccacttcataaaccacttccggttgaaaaacaagttcttattctttacgctttgacacatggcttcttggacagtgttccggttgatcaaatcttggattttgaagaagccctctatgactactttgatagccatcatgaggatatctttgaaacaatccgttcaactaaggatcttcctgaagaagctgtgcttaatgaagctatccaagctttcaaagatcaatcggaatacaaatag

SEQ ID NO: 8 - protein, 501 aa, Streptococcus thermophilus
LAINAQEISALIKKQIENFQPNFDVTETGVVTYIGDGIARARGLDNAMSGELLEFSNGVFGMAQNLESNDVGIIILGDFYTIREGDEVKRTGKIMEVPVGEALIGRVVNPLGQPIDGLGDIKTTATRPVEAPAPGVMQRKSVSEPLQTGLKAVDALVPIGRGQRELIIGDRQTGKTSVAIDAILNQKGQDVICIYVAIGQKESTVRTQVESLRKHGALDYTIVVTASASQPSPLLYIAPYAGVAMAEEFMYNGKHVLIVYDDLSKQAVAYRELSLLLRRPPGREAYPGDVFYLHSRLLERSAKLSDDLGGGSITALPIIQTQAGDISAYIATNVISITDGQIFLQENLFNSGIRPAIDAGSSVSRVGGSAQIKAMKKVAGTLRLDLASYRELEAFTQFGSDLDAATQAKLNRGRRTVEVLKQPLHKPLPVEKQVLILYALTHGFLDSVPVDQILDFEEALYDYFDSHHEDIFETIRSTKDLPEEAVLNEAIQAFKDQSEYK

SEQ ID NO: 9 - DNA, 1407 bp, Streptococcus thermophilus
  source 1..1407: mol_type = genomic DNA
atgagctcaggcaaaattgctcaggttgttggtcctgttgtagacgtagcgtttgcaactggcgataaacttcctgagattaacaatgcattggtcgtttacactgatgaagaaaagtctagacgtatcgtgctcgaagtagctcttgaacttggagaaggtgtggttcgtaccattgccatggaatctactgatggattgactcgtgggctagaagttctggacacaggtcgtccaatcagtgttcctgttggtaaagaaactcttggacgtgtctttaacgtgcttggagataccattgacatggaagcaccttttgcagatgatgcagagcgtgaaccaattcataaaaaagcacctaccttcgatgaattgtcaacaagtactgaaatccttgaaacagggattaaagttatcgacttgcttgccccttatcttaaaggtggtaaagtcggacttttcggtggtgccggtgttggtaagactgtccttattcaagagctgatccacaacattgctcaagaacacggtggcatttccgtgtttacgggtgttggggaacgttcacgtgaaggtaatgacctttactgggaaatgaaggaatctggcgttatcgaaaaaacagccatggtctttggtcaaatgaatgaaccacctggagcacgtatgcgtgttgcccttactggtttgactatcgctgaatatttccgtgatgttgaaggacaagacgtgcttctcttcattgataacatcttccgtttcactcaagcaggttctgaagtatcagcccttcttggtcgtatgccatcagccgttggttatcaacctacattggcaactgaaatgggtcaattgcaagaacgtatcacatcaactaaaaaaggttctgttacctcaatccaagctatctatgtcccggccgatgactacactgacccagcgccagcaacagcattcgctcacttggattcaacaactaaccttgaacgtaagttgacacaaatgggtatttatccagctgttgacccattggcatcaagctcacgtgccctttcacctgaaattgttggtgaagaacactatgctgttgcgactgaagttcaacgagtacttcaacgataccgtgaattgcaagatattatcgctatccttggtatggatgaattgtcggacgaagataaaacattggttggacgtgctcgtcgtatccaattcttcttgtcacaaaacttcaatgttgctgaacagtttacaggtcaaccaggttcttatgttccagttgctgaaactgttcgtggctttaaagaaatccttgaaggtaaatatgacaatcttcctgaagatgcctttcgtagcgtagggccaattgaggatgtagtagctaaagctaaagctatgggctactaa

SEQ ID NO: 10 - protein, 468 aa, Streptococcus thermophilus
MSSGKIAQVVGPVVDVAFATGDKLPEINNALVVYTDEEKSRRIVLEVALELGEGVVRTIAMESTDGLTRGLEVLDTGRPISVPVGKETLGRVFNVLGDTIDMEAPFADDAEREPIHKKAPTFDELSTSTEILETGIKVIDLLAPYLKGGKVGLFGGAGVGKTVLIQELIHNIAQEHGGISVFTGVGERSREGNDLYWEMKESGVIEKTAMVFGQMNEPPGARMRVALTGLTIAEYFRDVEGQDVLLFIDNIFRFTQAGSEVSALLGRMPSAVGYQPTLATEMGQLQERITSTKKGSVTSIQAIYVPADDYTDPAPATAFAHLDSTTNLERKLTQMGIYPAVDPLASSSRALSPEIVGEEHYAVATEVQRVLQRYRELQDIIAILGMDELSDEDKTLVGRARRIQFFLSQNFNVAEQFTGQPGSYVPVAETVRGFKEILEGKYDNLPEDAFRSVGPIEDVVAKAKAMGY

SEQ ID NO: 11 - DNA, 879 bp, Streptococcus thermophilus
  source 1..879: mol_type = genomic DNA
atggcaggctctctaagagaaatcaaagcaaaaattgcttcaattaagcaaacgagtcatattacaggagccatgcaaatggtttctgcttctaaattgacacgttctgagcaggctgctaaagatttccaaatctatgcctcaaaaattagacagatcacaacagatcttctacattcagaattggttaacggttcttcaaatccgatgttggatgcacgtccagttcgtaagtcagggtatattgtcattacttcagataagggattagttggaggatataattcaaccattcttaaagctgtcttggatatgattaaacgtgaccatgattctgaagatgaatatgctatcatctctattggtggaacaggttcagatttcttcaaagctcgtaacatgaatgttgcttttgaacttcgtggccttgaagatcaacctagtttcgatcaagtcgggaaaatcatttctaaagctgtaggaatgtatcaaaatgagctttttgatgaactttatgtgtgttacaatcatcatattaatagtttgtctcgtgaagttcgtgttgaaaaaatgcttccaattgctgattttgatcctaatgaatctgaaggccatgtattgaccaagtttgaattggaaccagatcgtgatactattttggatcaactcttgccacaatatgctgagagtcttatctacggtgctatcgtagatgccaaaacagctgagcatgctgctggtatgaccgcaatgcagactgccactgataatgctaagaaaataattaacgatttaacaattcaatacaaccgtgcacgtcaagcagccattactcaggaaatcactgagattgttggcggtgctagtgcacttgaatag

SEQ ID NO: 12 - protein, 292 aa, Streptococcus thermophilus
MAGSLREIKAKIASIKQTSHITGAMQMVSASKLTRSEQAAKDFQIYASKIRQITTDLLHSELVNGSSNPMLDARPVRKSGYIVITSDKGLVGGYNSTILKAVLDMIKRDHDSEDEYAIISIGGTGSDFFKARNMNVAFELRGLEDQPSFDQVGKIISKAVGMYQNELFDELYVCYNHHINSLSREVRVEKMLPIADFDPNESEGHVLTKFELEPDRDTILDQLLPQYAESLIYGAIVDAKTAEHAAGMTAMQTATDNAKKIINDLTIQYNRARQAAITQEITEIVGGASALE

SEQ ID NO: 13 - DNA, 537 bp, Streptococcus thermophilus
  source 1..537: mol_type = genomic DNA
atggataagaaaacacaagctcttgttgagcagtatgccagaagtctggtagaagtcgcttttgaacaagacgccgtgtcaacaatccaagaagaagtaaggcaaatcctaacagtttttgctgaaacaaatctaaaaaccttcttgtctcaagtaaatgtgacaagcgaggctaaaaaagaaagtttaagtttctttcaagagtcttgttcagtatacatgaacaattttcttgaggtaatttcactcaatgaccgagctaacattctttatgatgtcttgaaattggtccttgagctctttgatcaagaagacaacacttacgatgtcactgtgacatcagcaagttccttgtctgaagaacaaaaaactagacttttgacgatagtttcacaaaaatttgagattaagacacgtcgtttagtagaaaaaattgatgaggaactcattggaggattcgtcatcaaagcaaagaataagtttgttgacacgtcaattcgtagtcaattacaagcatttaaaatgaatttgaaatag

SEQ ID NO: 14 - protein, 178 aa, Streptococcus thermophilus
MDKKTQALVEQYARSLVEVAFEQDAVSTIQEEVRQILTVFAETNLKTFLSQVNVTSEAKKESLSFFQESCSVYMNNFLEVISLNDRANILYDVLKLVLELFDQEDNTYDVTVTSASSLSEEQKTRLLTIVSQKFEIKTRRLVEKIDEELIGGFVIKAKNKFVDTSIRSQLQAFKMNLK

SEQ ID NO: 15 - DNA, 447 bp, Streptococcus thermophilus
  source 1..447: mol_type = genomic DNA
atggcacaaatgaccgtacaagtggtaactccagatggtcttaaatatgaccaccatgccagctttatccacgcggttactaaagatggtcaaattggtattttgccaggccatattaacttgattgctccacttgaagtggatgagctcaaggttcgtcgtgtggatgacgagagtcacgtcgattggattgccgtaaacggtggtatcatcgaagttaaagatgatttcattactatcattgccaattcagcagaacgtgatcgcgacattgacgtttctcgtgccgaacgtgccaagcaacgtgccgaacgtgtcttggaagaagaaacaaaacgtgtcttggaagaagcaacaaaatctgatcgtaatgatgatgttcaacgtgctcagattgctctccgtcgagcacttaatcgtatcaatgtcggtacaaaaataagataa

SEQ ID NO: 16 - protein, 148 aa, Streptococcus thermophilus
MAQMTVQVVTPDGLKYDHHASFIHAVTKDGQIGILPGHINLIAPLEVDELKVRRVDDESHVDWIAVNGGIIEVKDDFITIIANSAERDRDIDVSRAERAKQRAERVLEEETKRVLEEATKSDRNDDVQRAQIALRRALNRINVGTKIR

SEQ ID NO: 17 - DNA, 20 bp, synthetic construct
  source 1..20: mol_type = other DNA; note = Fprimer
gacttgaagaaacagcgcgt

SEQ ID NO: 18 - DNA, 20 bp, synthetic construct
  source 1..20: mol_type = other DNA; note = Rprimer
taggtggaggcgttacagtg

SEQ ID NO: 19 - DNA, 20 bp, synthetic construct
  source 1..20: mol_type = other DNA; note = SNV F
tgaggtgaagatatggcaca

SEQ ID NO: 20 - DNA, 23 bp, synthetic construct
  source 1..23: mol_type = other DNA; note = SNV R
tctattacgttaccctacatttc

SEQ ID NO: 21 - DNA, 20 bp, synthetic construct
  source 1..20: mol_type = other DNA; note = 16S-F
caccggatacataccctcga

SEQ ID NO: 22 - DNA, 20 bp, synthetic construct
  source 1..20: mol_type = other DNA; note = 16S-R
tccctcacttcctgaacgtc

SEQ ID NO: 23 - DNA, 20 bp, synthetic construct
  source 1..20: mol_type = other DNA; note = LacI-F
atggtcgcaaagcttactga

SEQ ID NO: 24 - DNA, 20 bp, synthetic construct
  source 1..20: mol_type = other DNA; note = LacI-R
cagttcgtgacagacgaagc

SEQ ID NO: 25 - DNA, 20 bp, synthetic construct
  source 1..20: mol_type = other DNA; note = Insulinase-F
agcgattatctagtgcccca

SEQ ID NO: 26 - DNA, 20 bp, synthetic construct
  source 1..20: mol_type = other DNA; note = Insulinase-R
gcccttaatagctccaccac